European Patent Specification EP 3 787 688 B1, published October 30, 2024. Title: Compositions for Transfecting Resistant Cell Types. Applicant: Precision NanoSystems Inc. Precision NanoSystems Inc. The sequence listing filed with the application follows.

SEQUENCE LISTING (2 sequences)

SEQ ID NO: 1 - DNA, 5514 bp, Artificial
  Circular dsDNA pCX-EGFP
gtcgacattgattattgactagttattaatagtaatcaattacggggtcattagttcatagcccatatatggagttccgcgttacataacttacggtaaatggcccgcctggctgaccgcccaacgacccccgcccattgacgtcaataatgacgtatgttcccatagtaacgccaatagggactttccattgacgtcaatgggtggactatttacggtaaactgcccacttggcagtacatcaagtgtatcatatgccaagtacgccccctattgacgtcaatgacggtaaatggcccgcctggcattatgcccagtacatgaccttatgggactttcctacttggcagtacatctacgtattagtcatcgctattaccatgggtcgaggtgagccccacgttctgcttcactctccccatctcccccccctccccacccccaattttgtatttatttattttttaattattttgtgcagcgatgggggcggggggggggggggcgcgcgccaggcggggcggggcggggcgaggggcggggcggggcgaggcggagaggtgcggcggcagccaatcagagcggcgcgctccgaaagtttccttttatggcgaggcggcggcggcggcggccctataaaaagcgaagcgcgcggcgggcgggagtcgctgcgttgccttcgccccgtgccccgctccgcgccgcctcgcgccgcccgccccggctctgactgaccgcgttactcccacaggtgagcgggcgggacggcccttctcctccgggctgtaattagcgcttggtttaatgacggctcgtttcttttctgtggctgcgtgaaagccttaaagggctccgggagggccctttgtgcgggggggagcggctcggggggtgcgtgcgtgtgtgtgtgcgtggggagcgccgcgtgcggcccgcgctgcccggcggctgtgagcgctgcgggcgcggcgcggggctttgtgcgctccgcgtgtgcgcgaggggagcgcggccgggggcggtgccccgcggtgcgggggggctgcgaggggaacaaaggctgcgtgcggggtgtgtgcgtgggggggtgagcagggggtgtgggcgcggcggtcgggctgtaacccccccctgcacccccctccccgagttgctgagcacggcccggcttcgggtgcggggctccgtacggggcgtggcgcggggctcgccgtgccgggcggggggtggcggcaggtgggggtgccgggcggggcggggccgcctcgggccggggagggctcgggggaggggcgcggcggcccccggagcgccggcggctgtcgaggcgcggcgagccgcagccattgccttttatggtaatcgtgcgagagggcgcagggacttcctttgtcccaaatctgtgcggagccgaaatctgggaggcgccgccgcaccccctctagcgggcgcggggcgaagcggtgcggcgccggcaggaaggaactgggcggggagggccttcgtgcgtcgccgcgccgccgtccccttctccctctccagcctcggggctgtccgcggggggacggctgccttcgggggggacggggcagggcggggttcggcttctggcgtgtgaccggcggctctagagcctctgctaaccatgttcatgccttcttctttttcctacagctcctgggcaacgtgctggttattgtgctgtctcatcattttggcaaagaattcgccaccatggtgagcaagggcgaggagctgttcaccggggtggtgcccatcctggtcgagctggacggcgacgtgaacggccacaagttcagcgtgtccggcgagggcgagggcgatgccacctacggcaagctgaccctgaagttcatctgcaccaccggcaagctgcccgtgccctggcccaccctcgtgaccaccctgacctacggcgtgcagtgcttcagccgctaccccgaccacatgaagcagcacgacttcttcaagtccgccatgcccgaaggctacgtccaggagcgcaccatcttcttcaaggacgacggcaactacaagacccgcgccgaggtgaagttcgagggcgacaccctggtgaaccgcatcgagctgaagggcatcgacttcaaggaggacggcaacatcctggggcacaagctggagtacaactacaacagccacaacgtctatatcatggccgacaagcagaagaacggcatcaaggtgaacttcaagatccgccacaacatcgaggacggcagcgtgcagctcgccgaccactaccagcagaacacccccatcggcgacggccccgtgctgctgcccgacaaccactacctgagcacccagtccgccctgagcaaagaccccaacgagaagcgcgatcacatggtcctgctggagttcgtgaccgccgccgggatcactcacggcatggacgagctgtacaagtaagaattcactcctcaggtgcaggctgcctatcagaaggtggtggctggtgtggccaatgccctggctcacaaataccactgagatctttttccctctgccaaaaattatggggacatcatgaagccccttgagcatctgacttctggctaataaaggaaatttattttcattgcaatagtgtgttggaattttttgtgtctctcactcggaaggacatatgggagggcaaatcatttaaaacatcagaatgagtatttggtttagagtttggcaacatatgccatatgctggctgccatgaacaaaggtggctataaagaggtcatcagtatatgaaacagccccctgctgtccattccttattccatagaaaagccttgacttgaggttagattttttttatattttgttttgtgttatttttttctttaacatccctaaaattttccttacatgttttactagccagatttttcctcctctcctgactactcccagtcatagctgtccctcttctcttatgaagatccctcgacctgcagcccaagcttggcgtaatcatggtcatagctgtttcctgtgtgaaattgttatccgctcacaattccacacaacatacgagccggaagcataaagtgtaaagcctggggtgcctaatgagtgagctaactcacattaattgcgttgcgctcactgcccgctttccagtcgggaaacctgtcgtgccagcggatccgcatctcaattagtcagcaaccatagtcccgcccctaactccgcccatcccgcccctaactccgcccagttccgcccattctccgccccatggctgactaattttttttatttatgcagaggccgaggccgcctcggcctctgagctattccagaagtagtgaggaggcttttttggaggcctaggcttttgcaaaaagctaacttgtttattgcagcttataatggttacaaataaagcaatagcatcacaaatttcacaaataaagcatttttttcactgcattctagttgtggtttgtccaaactcatcaatgtatcttatcatgtctggatccgctgcattaatgaatcggccaacgcgcggggagaggcggtttgcgtattgggcgctcttccgcttcctcgctcactgactcgctgcgctcggtcgttcggctgcggcgagcggtatcagctcactcaaaggcggtaatacggttatccacagaatcaggggataacgcaggaaagaacatgtgagcaaaaggccagcaaaaggccaggaaccgtaaaaaggccgcgttgctggcgtttttccataggctccgcccccctgacgagcatcacaaaaatcgacgctcaagtcagaggtggcgaaacccgacaggactataaagataccaggcgtttccccctggaagctccctcgtgcgctctcctgttccgaccctgccgcttaccggatacctgtccgcctttctcccttcgggaagcgtggcgctttctcaatgctcacgctgtaggtatctcagttcggtgtaggtcgttcgctccaagctgggctgtgtgcacgaaccccccgttcagcccgaccgctgcgccttatccggtaactatcgtcttgagtccaacccggtaagacacgacttatcgccactggcagcagccactggtaacaggattagcagagcgaggtatgtaggcggtgctacagagttcttgaagtggtggcctaactacggctacactagaaggacagtatttggtatctgcgctctgctgaagccagttaccttcggaaaaagagttggtagctcttgatccggcaaacaaaccaccgctggtagcggtggtttttttgtttgcaagcagcagattacgcgcagaaaaaaaggatctcaagaagatcctttgatcttttctacggggtctgacgctcagtggaacgaaaactcacgttaagggattttggtcatgagattatcaaaaaggatcttcacctagatccttttaaattaaaaatgaagttttaaatcaatctaaagtatatatgagtaaacttggtctgacagttaccaatgcttaatcagtgaggcacctatctcagcgatctgtctatttcgttcatccatagttgcctgactccccgtcgtgtagataactacgatacgggagggcttaccatctggccccagtgctgcaatgataccgcgagacccacgctcaccggctccagatttatcagcaataaaccagccagccggaagggccgagcgcagaagtggtcctgcaactttatccgcctccatccagtctattaattgttgccgggaagctagagtaagtagttcgccagttaatagtttgcgcaacgttgttgccattgctacaggcatcgtggtgtcacgctcgtcgtttggtatggcttcattcagctccggttcccaacgatcaaggcgagttacatgatcccccatgttgtgcaaaaaagcggttagctccttcggtcctccgatcgttgtcagaagtaagttggccgcagtgttatcactcatggttatggcagcactgcataattctcttactgtcatgccatccgtaagatgcttttctgtgactggtgagtactcaaccaagtcattctgagaatagtgtatgcggcgaccgagttgctcttgcccggcgtcaatacgggataataccgcgccacatagcagaactttaaaagtgctcatcattggaaaacgttcttcggggcgaaaactctcaaggatcttaccgctgttgagatccagttcgatgtaacccactcgtgcacccaactgatcttcagcatcttttactttcaccagcgtttctgggtgagcaaaaacaggaaggcaaaatgccgcaaaaaagggaataagggcgacacggaaatgttgaatactcatactcttcctttttcaatattattgaagcatttatcagggttattgtctcatgagcggatacatatttgaatgtatttagaaaaataaacaaataggggttccgcgcacatttccccgaaaagtgccacctg

SEQ ID NO: 2 - DNA, 966 bp, Artificial
  mRNA eGFP ORF
  misc_feature (721)..(846): n is a, c, g, t or u
atggtgagcaagggcgaggagctgttcaccggggtggtgcccatcctggtcgagctggacggcgacgtaaacggccacaagttcagcgtgtccggcgagggcgagggcgatgccacctacggcaagctgaccctgaagttcatctgcaccaccggcaagctgcccgtgccctggcccaccctcgtgaccaccctgacctacggcgtgcagtgcttcagccgctaccccgaccacatgaagcagcacgacttcttcaagtccgccatgcccgaaggctacgtccaggagcgcaccatcttcttcaaggacgacggcaactacaagacccgcgccgaggtgaagttcgagggcgacaccctggtgaaccgcatcgagctgaagggcatcgacttcaaggaggacggcaacatcctggggcacaagctggagtacaactacaacagccacaacgtctatatcatggccgacaagcagaagaacggcatcaaggtgaacttcaagatccgccacaacatcgaggacggcagcgtgcagctcgccgaccactaccagcagaacacccccatcggcgacggccccgtgctgctgcccgacaaccactacctgagcacccagtccgccctgagcaaagaccccaacgagaagcgcgatcacatggtcctgctggagttcgtgaccgccgccgggatcactctcggcatggacgagctgtacaagtaannnnnnnnnnnnnnnnnnnnnnnnnnnnnnnnnnnnnnnnnnnnnnnnnnnnnnnnnnnnnnnnnnnnnnnnnnnnnnnnnnnnnnnnnnnnnnnnnnnnnnnnnnnnnnnnnnnnnnnnnnnnnnaaaaaaaaaaaaaaaaaaaaaaaaaaaaaaaaaaaaaaaaaaaaaaaaaaaaaaaaaaaaaaaaaaaaaaaaaaaaaaaaaaaaaaaaaaaaaaaaaaaaaaaaaaaaaaaaaaaaaaaa